European Patent Specification EP 3 596 222 B1, published April 12, 2023. Title: ADENO-ASSOCIATED VIRUS VECTOR DELIVERY OF MUSCLE SPECIFIC MICRO-DYSTROPHIN TO TREAT MUSCULAR DYSTROPHY. Applicant: RESEARCH INSTITUTE AT NATIONWIDE CHILDREN'S HOSPITAL. The sequence listing filed with the application follows.

SEQUENCE LISTING (5 sequences)

SEQ ID NO: 1 - DNA, 3579 bp, Homo sapiens
atgctgtggtgggaggaggtggaggattgttatgaaagggaggacgtgcagaagaagacttttaccaagtgggtgaacgctcagttcagcaaatttgggaagcagcacatcgagaatctgttttccgacctgcaggatgggagacggctgctggatctgctggaaggactgactggccagaagctgcccaaagagaaggggagcactagggtgcacgccctgaacaacgtgaacaaagctctgagagtgctgcagaacaacaacgtggatctggtgaatattggcagtactgatatcgtggacgggaaccacaaactgacactgggcctgatctggaacattattctgcactggcaggtgaaaaatgtgatgaagaacatcatggccgggctgcagcagaccaattccgagaagatcctgctgtcttgggtgcggcagagcacccgcaactatccccaggtgaacgtgattaacttcactacatcctggagcgacgggctggccctgaatgctctgattcacagccacaggcctgatctgttcgactggaatagcgtggtgtgccagcagtctgccacacagcgcctggaacatgccttcaatatcgctcggtaccagctggggatcgaaaaactgctggacccagaggatgtggacactacatacccagataaaaagtctattctgatgtacattactagcctgttccaggtgctgccacagcaggtgtctattgaagccattcaggaggtggaaatgctgccccgcccccccaaagtgactaaagaggagcattttcagctgcatcatcagatgcattacagccagcagattaccgtgagcctggctcagggatatgagcgcaccagtagtccaaaaccacggttcaagtcctacgcttatacccaggctgcctacgtgacaactagcgaccctactagatccccctttccatcccagcacctggaggccccagaggacaagagctttgggtccagcctgatggaaagcgaggtgaatctggatcggtaccagacagccctggaggaggtgctgagctggctgctgagtgctgaagacacactgcaggcccagggcgaaatttccaatgacgtggaagtggtgaaggatcagttccacacacacgagggctatatgatggacctgacagctcaccaggggcgcgtgggcaatatcctgcagctgggctctaaactgatcggcaccgggaaactgagtgaggacgaggaaacagaagtgcaggagcagatgaacctgctgaacagccgctgggagtgtctgagagtggctagtatggagaagcagtccaacctgcaccgggtgctgatggacctgcagaaccagaaactgaaagagctgaacgactggctgacaaagactgaggaacgcacaaggaagatggaggaggagccactgggacccgacctggaggatctgaagagacaggtgcagcagcataaggtgctgcaggaggatctggaacaggagcaggtgcgggtgaactccctgacacatatggtggtggtggtggacgaatctagtggagatcacgccaccgccgccctggaggaacagctgaaggtgctgggggaccggtgggccaacatttgccggtggaccgaggacaggtgggtgctgctgcaggacatcctgctgaaatggcagaggctgaccgaggagcagtgtctgtttagtgcttggctgagcgagaaagaggacgccgtgaacaagatccacacaaccggctttaaggatcagaacgaaatgctgtctagcctgcagaaactggctgtgctgaaggccgatctggagaaaaagaagcagagcatgggcaaactgtatagcctgaaacaggacctgctgagcaccctgaagaacaagagcgtgacccagaagacagaagcctggctggataactttgcccgctgctgggacaacctggtgcagaaactggagaaaagtacagctcagatctctcaggctgtgaccacaacccagcctagcctgacccagacaaccgtgatggaaaccgtgaccaccgtgacaacccgcgaacagatcctggtgaaacatgcccaggaagagctgccacctccacctccccagaagaagagaaccctggagcggctgcaggagctgcaggaagccactgacgaactggacctgaagctgaggcaggccgaagtgattaaggggtcttggcagcctgtgggcgatctgctgattgattccctgcaggaccacctggaaaaggtgaaggctctgagaggcgaaattgctccactgaaggagaacgtgagtcatgtgaacgatctggctagacagctgacaacactgggcatccagctgagcccatacaatctgagcacactggaggacctgaataccaggtggaagctgctgcaggtggctgtggaagaccgggtgcggcagctgcatgaggcccatcgcgacttcggaccagccagccagcactttctgagcacatccgtgcaggggccctgggagagggccatttctcccaacaaggtgccctactatattaatcacgagacccagaccacttgttgggaccatcccaagatgacagaactgtaccagtccctggccgatctgaacaacgtgaggtttagcgcttacagaaccgctatgaagctgagacggctgcagaaggccctgtgcctggatctgctgtccctgtccgccgcctgcgatgccctggatcagcataatctgaagcagaacgatcagccaatggatatcctgcagatcatcaactgcctgaccactatctacgacaggctggagcaggagcacaacaacctggtgaacgtgcctctgtgcgtggatatgtgcctgaactggctgctgaacgtgtatgacactgggcgcaccggccggatcagagtgctgagttttaaaactgggattatctccctgtgtaaggcccacctggaggacaagtacaggtacctgttcaagcaggtggctagtagcactggattttgtgaccagcgccgcctgggactgctgctgcatgatagtatccagattcctagacagctgggagaggtggctagtttcggaggatctaacatcgaacccagcgtgcgcagctgtttccagtttgccaataacaaacctgaaatcgaggctgctctgttcctggattggatgcgcctggaaccacagagcatggtgtggctgcctgtgctgcacagagtggctgccgccgaaactgccaagcaccaggctaaatgcaacatctgcaaggaatgtcccattatcggctttcgctacaggagtctgaaacattttaactacgatatttgccagagctgcttcttttccggaagagtggccaaaggacacaagatgcactaccctatggtggaatattgcaccccaactacatctggcgaagatgtgcgcgattttgccaaggtgctgaagaataagtttcggactaagaggtacttcgccaagcacccccgcatggggtatctgccagtgcagacagtgctggaaggagacaatatggagaccgatacaatgtga

SEQ ID NO: 2 - DNA, 810 bp, Adeno-associated virus
gtttaaacaagcttgcatgtctaagctagacccttcagattaaaaataactgaggtaagggcctgggtaggggaggtggtgtgagacgctcctgtctctcctctatctgcccatcggccctttggggaggaggaatgtgcccaaggactaaaaaaaggccatggagccagaggggcgagggcaacagacctttcatgggcaaaccttggggccctgctgtctagcatgccccactacgggtctaggctgcccatgtaaggaggcaaggcctggggacacccgagatgcctggttataattaacccagacatgtggctgcccccccccccccaacacctgctgcctctaaaaataaccctgtccctggtggatcccctgcatgcgaagatcttcgaacaaggctgtgggggactgagggcaggctgtaacaggcttgggggccagggcttatacgtgcctgggactcccaaagtattactgttccatgttcccggcgaagggccagctgtcccccgccagctagactcagcacttagtttaggaaccagtgagcaagtcagcccttggggcagcccatacaaggccatggggctgggcaagctgcacgcctgggtccggggtgggcacggtgcccgggcaacgagctgaaagctcatctgctctcaggggcccctccctggggacagcccctcctggctagtcacaccctgtaggctcctctatataacccaggggcacaggggctgccctcattctaccaccacctccacagcacagacagacactcaggagccagccagcggcgcgccc

SEQ ID NO: 3 - DNA, 8611 bp, Adeno-associated virus
gcccaatacgcaaaccgcctctccccgcgcgttggccgattcattaatgcagctggcgcgctcgctcgctcactgaggccgcccgggcaaagcccgggcgtcgggcgacctttggtcgcccggcctcagtgagcgagcgagcgcgcagagagggagtggccaactccatcactaggggttccttgtagttaatgattaacccgccatgctaattatctacgtagccatgtctagagtttaaacaagcttgcatgtctaagctagacccttcagattaaaaataactgaggtaagggcctgggtaggggaggtggtgtgagacgctcctgtctctcctctatctgcccatcggccctttggggaggaggaatgtgcccaaggactaaaaaaaggccatggagccagaggggcgagggcaacagacctttcatgggcaaaccttggggccctgctgtctagcatgccccactacgggtctaggctgcccatgtaaggaggcaaggcctggggacacccgagatgcctggttataattaacccagacatgtggctgcccccccccccccaacacctgctgcctctaaaaataaccctgtccctggtggatcccctgcatgcgaagatcttcgaacaaggctgtgggggactgagggcaggctgtaacaggcttgggggccagggcttatacgtgcctgggactcccaaagtattactgttccatgttcccggcgaagggccagctgtcccccgccagctagactcagcacttagtttaggaaccagtgagcaagtcagcccttggggcagcccatacaaggccatggggctgggcaagctgcacgcctgggtccggggtgggcacggtgcccgggcaacgagctgaaagctcatctgctctcaggggcccctccctggggacagcccctcctggctagtcacaccctgtaggctcctctatataacccaggggcacaggggctgccctcattctaccaccacctccacagcacagacagacactcaggagccagccagcggcgcgcccaggtaagtttagtctttttgtcttttatttcaggtcccggatccggtggtggtgcaaatcaaagaactgctcctcagtggatgttgcctttacttctaggcctgtacggaagtgttacttctgctctaaaagctgcggaattgtacccgcggccgccaccatgctgtggtgggaggaggtggaggattgttatgaaagggaggacgtgcagaagaagacttttaccaagtgggtgaacgctcagttcagcaaatttgggaagcagcacatcgagaatctgttttccgacctgcaggatgggagacggctgctggatctgctggaaggactgactggccagaagctgcccaaagagaaggggagcactagggtgcacgccctgaacaacgtgaacaaagctctgagagtgctgcagaacaacaacgtggatctggtgaatattggcagtactgatatcgtggacgggaaccacaaactgacactgggcctgatctggaacattattctgcactggcaggtgaaaaatgtgatgaagaacatcatggccgggctgcagcagaccaattccgagaagatcctgctgtcttgggtgcggcagagcacccgcaactatccccaggtgaacgtgattaacttcactacatcctggagcgacgggctggccctgaatgctctgattcacagccacaggcctgatctgttcgactggaatagcgtggtgtgccagcagtctgccacacagcgcctggaacatgccttcaatatcgctcggtaccagctggggatcgaaaaactgctggacccagaggatgtggacactacatacccagataaaaagtctattctgatgtacattactagcctgttccaggtgctgccacagcaggtgtctattgaagccattcaggaggtggaaatgctgccccgcccccccaaagtgactaaagaggagcattttcagctgcatcatcagatgcattacagccagcagattaccgtgagcctggctcagggatatgagcgcaccagtagtccaaaaccacggttcaagtcctacgcttatacccaggctgcctacgtgacaactagcgaccctactagatccccctttccatcccagcacctggaggccccagaggacaagagctttgggtccagcctgatggaaagcgaggtgaatctggatcggtaccagacagccctggaggaggtgctgagctggctgctgagtgctgaagacacactgcaggcccagggcgaaatttccaatgacgtggaagtggtgaaggatcagttccacacacacgagggctatatgatggacctgacagctcaccaggggcgcgtgggcaatatcctgcagctgggctctaaactgatcggcaccgggaaactgagtgaggacgaggaaacagaagtgcaggagcagatgaacctgctgaacagccgctgggagtgtctgagagtggctagtatggagaagcagtccaacctgcaccgggtgctgatggacctgcagaaccagaaactgaaagagctgaacgactggctgacaaagactgaggaacgcacaaggaagatggaggaggagccactgggacccgacctggaggatctgaagagacaggtgcagcagcataaggtgctgcaggaggatctggaacaggagcaggtgcgggtgaactccctgacacatatggtggtggtggtggacgaatctagtggagatcacgccaccgccgccctggaggaacagctgaaggtgctgggggaccggtgggccaacatttgccggtggaccgaggacaggtgggtgctgctgcaggacatcctgctgaaatggcagaggctgaccgaggagcagtgtctgtttagtgcttggctgagcgagaaagaggacgccgtgaacaagatccacacaaccggctttaaggatcagaacgaaatgctgtctagcctgcagaaactggctgtgctgaaggccgatctggagaaaaagaagcagagcatgggcaaactgtatagcctgaaacaggacctgctgagcaccctgaagaacaagagcgtgacccagaagacagaagcctggctggataactttgcccgctgctgggacaacctggtgcagaaactggagaaaagtacagctcagatctctcaggctgtgaccacaacccagcctagcctgacccagacaaccgtgatggaaaccgtgaccaccgtgacaacccgcgaacagatcctggtgaaacatgcccaggaagagctgccacctccacctccccagaagaagagaaccctggagcggctgcaggagctgcaggaagccactgacgaactggacctgaagctgaggcaggccgaagtgattaaggggtcttggcagcctgtgggcgatctgctgattgattccctgcaggaccacctggaaaaggtgaaggctctgagaggcgaaattgctccactgaaggagaacgtgagtcatgtgaacgatctggctagacagctgacaacactgggcatccagctgagcccatacaatctgagcacactggaggacctgaataccaggtggaagctgctgcaggtggctgtggaagaccgggtgcggcagctgcatgaggcccatcgcgacttcggaccagccagccagcactttctgagcacatccgtgcaggggccctgggagagggccatttctcccaacaaggtgccctactatattaatcacgagacccagaccacttgttgggaccatcccaagatgacagaactgtaccagtccctggccgatctgaacaacgtgaggtttagcgcttacagaaccgctatgaagctgagacggctgcagaaggccctgtgcctggatctgctgtccctgtccgccgcctgcgatgccctggatcagcataatctgaagcagaacgatcagccaatggatatcctgcagatcatcaactgcctgaccactatctacgacaggctggagcaggagcacaacaacctggtgaacgtgcctctgtgcgtggatatgtgcctgaactggctgctgaacgtgtatgacactgggcgcaccggccggatcagagtgctgagttttaaaactgggattatctccctgtgtaaggcccacctggaggacaagtacaggtacctgttcaagcaggtggctagtagcactggattttgtgaccagcgccgcctgggactgctgctgcatgatagtatccagattcctagacagctgggagaggtggctagtttcggaggatctaacatcgaacccagcgtgcgcagctgtttccagtttgccaataacaaacctgaaatcgaggctgctctgttcctggattggatgcgcctggaaccacagagcatggtgtggctgcctgtgctgcacagagtggctgccgccgaaactgccaagcaccaggctaaatgcaacatctgcaaggaatgtcccattatcggctttcgctacaggagtctgaaacattttaactacgatatttgccagagctgcttcttttccggaagagtggccaaaggacacaagatgcactaccctatggtggaatattgcaccccaactacatctggcgaagatgtgcgcgattttgccaaggtgctgaagaataagtttcggactaagaggtacttcgccaagcacccccgcatggggtatctgccagtgcagacagtgctggaaggagacaatatggagaccgatacaatgtgagcggccgcaataaaagatctttattttcattagatctgtgtgttggttttttgtgtgtctagagcatggctacgtagataagtagcatggcgggttaatcattaactacaaggaacccctagtgatggagttggccactccctctctgcgcgctcgctcgctcactgaggccgggcgaccaaaggtcgcccgacgcccgggctttgcccgggcggcctcagtgagcgagcgagcgcgccagctggcgtaatagcgaagaggcccgcaccgatcgcccttcccaacagttgcgcagcctgaatggcgaatggaagttccagacgattgagcgtcaaaatgtaggtatttccatgagcgtttttcctgttgcaatggctggcggtaatattgttctggatattaccagcaaggccgatagtttgagttcttctactcaggcaagtgatgttattactaatcaaagaagtattgcgacaacggttaatttgcgtgatggacagactcttttactcggtggcctcactgattataaaaacacttctcaggattctggcgtaccgttcctgtctaaaatccctttaatcggcctcctgtttagctcccgctctgattctaacgaggaaagcacgttatacgtgctcgtcaaagcaaccatagtacgcgccctgtagcggcgcattaagcgcggcgggtgtggtggttacgcgcagcgtgaccgctacacttgccagcgccctagcgcccgctcctttcgctttcttcccttcctttctcgccacgttcgccggctttccccgtcaagctctaaatcgggggctccctttagggttccgatttagtgatttacggcacctcgaccccaaaaaacttgattagggtgatggttcacgtagtgggccatcgccctgatagacggtttttcgccctttgacgttggagtccacgttctttaatagtggactcttgttccaaactggaacaacactcaaccctatctcggtctattcttttgatttataagggattttgccgatttcggcctattggttaaaaaatgagctgatttaacaaaaatttaacgcgaattttaacaaaatattaacgtttacaatttaaatatttgcttatacaatcttcctgtttttggggcttttctgattatcaaccggggtacatatgattgacatgctagttttacgattaccgttcatcgattctcttgtttgctccagactctcaggcaatgacctgatagcctttgtagagacctctcaaaaatagctaccctctccggcatgaatttatcagctagaacggttgaatatcatattgatggtgatttgactgtctccggcctttctcacccgtttgaatctttacctacacattactcaggcattgcatttaaaatatatgagggttctaaaaatttttatccttgcgttgaaataaaggcttctcccgcaaaagtattacagggtcataatgtttttggtacaaccgatttagctttatgctctgaggctttattgcttaattttgctaattctttgccttgcctgtatgatttattggatgttggaagttcctgatgcggtattttctccttacgcatctgtgcggtatttcacaccgcatatggtgcactctcagtacaatctgctctgatgccgcatagttaagccagccccgacacccgccaacacccgctgacgcgccctgacgggcttgtctgctcccggcatccgcttacagacaagctgtgaccgtctccgggagctgcatgtgtcagaggttttcaccgtcatcaccgaaacgcgcgagacgaaagggcctcgtgatacgcctatttttataggttaatgtcatgataataatggtttcttagacgtcaggtggcacttttcggggaaatgtgcgcggaacccctatttgtttatttttctaaatacattcaaatatgtatccgctcatgagacaataaccctgataaatgcttcaataatattgaaaaaggaagagtatgagtattcaacatttccgtgtcgcccttattcccttttttgcggcattttgccttcctgtttttgctcacccagaaacgctggtgaaagtaaaagatgctgaagatcagttgggtgcacgagtgggttacatcgaactggatctcaacagcggtaagatccttgagagttttcgccccgaagaacgttttccaatgatgagcacttttaaagttctgctatgtggcgcggtattatcccgtattgacgccgggcaagagcaactcggtcgccgcatacactattctcagaatgacttggttgagtactcaccagtcacagaaaagcatcttacggatggcatgacagtaagagaattatgcagtgctgccataaccatgagtgataacactgcggccaacttacttctgacaacgatcggaggaccgaaggagctaaccgcttttttgcacaacatgggggatcatgtaactcgccttgatcgttgggaaccggagctgaatgaagccataccaaacgacgagcgtgacaccacgatgcctgtagcaatggcaacaacgttgcgcaaactattaactggcgaactacttactctagcttcccggcaacaattaatagactggatggaggcggataaagttgcaggaccacttctgcgctcggcccttccggctggctggtttattgctgataaatctggagccggtgagcgtgggtctcgcggtatcattgcagcactggggccagatggtaagccctcccgtatcgtagttatctacacgacggggagtcaggcaactatggatgaacgaaatagacagatcgctgagataggtgcctcactgattaagcattggtaactgtcagaccaagtttactcatatatactttagattgatttaaaacttcatttttaatttaaaaggatctaggtgaagatcctttttgataatctcatgaccaaaatcccttaacgtgagttttcgttccactgagcgtcagaccccgtagaaaagatcaaaggatcttcttgagatcctttttttctgcgcgtaatctgctgcttgcaaacaaaaaaaccaccgctaccagcggtggtttgtttgccggatcaagagctaccaactctttttccgaaggtaactggcttcagcagagcgcagataccaaatactgtccttctagtgtagccgtagttaggccaccacttcaagaactctgtagcaccgcgtacatacctcgctctgctaatcctgttaccagtggctgctgccagtggcgataagtcgtgtcttaccgggttggactcaagacgatagttaccggataaggcgcagcggtcgggctgaacggggggttcgtgcacacagcccagcttggagcgaacgacctacaccgaactgagatacctacagcgtgagctatgagaaagcgccacgcttcccgaagggagaaaggcggacaggtatccggtaagcggcagggtcggaacaggagagcgcacgagggagcttccagggggaaacgcctggtatctttatagtcctgtcgggtttcgccacctctgacttgagcgtcgatttttgtgatgctcgtcaggggggcggagcctatggaaaaacgccagcaacgcggcctttttacggttcctggccttttgctggccttttgctcacatgttctttcctgcgttatcccctgattctgtggataaccgtattaccgggtttgagtgagctgataccgctcgccgcagccgaacgaccgagcgcagcgagtcagtgagcgaccaagcggaagagc

SEQ ID NO: 4 - DNA, 564 bp, Adeno-associated virus
cagccactatgggtctaggctgcccatgtaaggaggcaaggcctggggacacccgagatgcctggttataattaacccagacatgtggctgctccccccccccaacacctgctgcctgagcctcacccccaccccggtgcctgggtcttaggctctgtacaccatggaggagaagctcgctctaaaaataaccctgtccctggtgggctgtgggggactgagggcaggctgtaacaggcttgggggccagggcttatacgtgcctgggactcccaaagtattactgttccatgttcccggcgaagggccagctgtcccccgccagctagactcagcacttagtttaggaaccagtgagcaagtcagcccttggggcagcccatacaaggccatggggctgggcaagctgcacgcctgggtccggggtgggcacggtgcccgggcaacgagctgaaagctcatctgctctcaggggcccctccctggggacagcccctcctggctagtcacaccctgtaggctcctctatataacccaggggcacaggggctgcccccgggtcac

SEQ ID NO: 5 - DNA, 8409 bp, Adeno associated virus
gcccaatacgcaaaccgcctctccccgcgcgttggccgattcattaatgcagctggcgcgctcgctcgctcactgaggccgcccgggcaaagcccgggcgtcgggcgacctttggtcgcccggcctcagtgagcgagcgagcgcgcagagagggagtggccaactccatcactaggggttccttgtagttaatgattaacccgccatgctaattatctacgtagccatgtctagacagccactatgggtctaggctgcccatgtaaggaggcaaggcctggggacacccgagatgcctggttataattaacccagacatgtggctgctccccccccccaacacctgctgcctgagcctcacccccaccccggtgcctgggtcttaggctctgtacaccatggaggagaagctcgctctaaaaataaccctgtccctggtgggctgtgggggactgagggcaggctgtaacaggcttgggggccagggcttatacgtgcctgggactcccaaagtattactgttccatgttcccggcgaagggccagctgtcccccgccagctagactcagcacttagtttaggaaccagtgagcaagtcagcccttggggcagcccatacaaggccatggggctgggcaagctgcacgcctgggtccggggtgggcacggtgcccgggcaacgagctgaaagctcatctgctctcaggggcccctccctggggacagcccctcctggctagtcacaccctgtaggctcctctatataacccaggggcacaggggctgcccccgggtcaccaccacctccacagcacagacagacactcaggagccagccagccaggtaagtttagtctttttgtcttttatttcaggtcccggatccggtggtggtgcaaatcaaagaactgctcctcagtggatgttgcctttacttctaggcctgtacggaagtgttacttctgctctaaaagctgcggaattgtacccgcggccgccaccatgctgtggtgggaggaggtggaggattgttatgaaagggaggacgtgcagaagaagacttttaccaagtgggtgaacgctcagttcagcaaatttgggaagcagcacatcgagaatctgttttccgacctgcaggatgggagacggctgctggatctgctggaaggactgactggccagaagctgcccaaagagaaggggagcactagggtgcacgccctgaacaacgtgaacaaagctctgagagtgctgcagaacaacaacgtggatctggtgaatattggcagtactgatatcgtggacgggaaccacaaactgacactgggcctgatctggaacattattctgcactggcaggtgaaaaatgtgatgaagaacatcatggccgggctgcagcagaccaattccgagaagatcctgctgtcttgggtgcggcagagcacccgcaactatccccaggtgaacgtgattaacttcactacatcctggagcgacgggctggccctgaatgctctgattcacagccacaggcctgatctgttcgactggaatagcgtggtgtgccagcagtctgccacacagcgcctggaacatgccttcaatatcgctcggtaccagctggggatcgaaaaactgctggacccagaggatgtggacactacatacccagataaaaagtctattctgatgtacattactagcctgttccaggtgctgccacagcaggtgtctattgaagccattcaggaggtggaaatgctgccccgcccccccaaagtgactaaagaggagcattttcagctgcatcatcagatgcattacagccagcagattaccgtgagcctggctcagggatatgagcgcaccagtagtccaaaaccacggttcaagtcctacgcttatacccaggctgcctacgtgacaactagcgaccctactagatccccctttccatcccagcacctggaggccccagaggacaagagctttgggtccagcctgatggaaagcgaggtgaatctggatcggtaccagacagccctggaggaggtgctgagctggctgctgagtgctgaagacacactgcaggcccagggcgaaatttccaatgacgtggaagtggtgaaggatcagttccacacacacgagggctatatgatggacctgacagctcaccaggggcgcgtgggcaatatcctgcagctgggctctaaactgatcggcaccgggaaactgagtgaggacgaggaaacagaagtgcaggagcagatgaacctgctgaacagccgctgggagtgtctgagagtggctagtatggagaagcagtccaacctgcaccgggtgctgatggacctgcagaaccagaaactgaaagagctgaacgactggctgacaaagactgaggaacgcacaaggaagatggaggaggagccactgggacccgacctggaggatctgaagagacaggtgcagcagcataaggtgctgcaggaggatctggaacaggagcaggtgcgggtgaactccctgacacatatggtggtggtggtggacgaatctagtggagatcacgccaccgccgccctggaggaacagctgaaggtgctgggggaccggtgggccaacatttgccggtggaccgaggacaggtgggtgctgctgcaggacatcctgctgaaatggcagaggctgaccgaggagcagtgtctgtttagtgcttggctgagcgagaaagaggacgccgtgaacaagatccacacaaccggctttaaggatcagaacgaaatgctgtctagcctgcagaaactggctgtgctgaaggccgatctggagaaaaagaagcagagcatgggcaaactgtatagcctgaaacaggacctgctgagcaccctgaagaacaagagcgtgacccagaagacagaagcctggctggataactttgcccgctgctgggacaacctggtgcagaaactggagaaaagtacagctcagatctctcaggctgtgaccacaacccagcctagcctgacccagacaaccgtgatggaaaccgtgaccaccgtgacaacccgcgaacagatcctggtgaaacatgcccaggaagagctgccacctccacctccccagaagaagagaaccctggagcggctgcaggagctgcaggaagccactgacgaactggacctgaagctgaggcaggccgaagtgattaaggggtcttggcagcctgtgggcgatctgctgattgattccctgcaggaccacctggaaaaggtgaaggctctgagaggcgaaattgctccactgaaggagaacgtgagtcatgtgaacgatctggctagacagctgacaacactgggcatccagctgagcccatacaatctgagcacactggaggacctgaataccaggtggaagctgctgcaggtggctgtggaagaccgggtgcggcagctgcatgaggcccatcgcgacttcggaccagccagccagcactttctgagcacatccgtgcaggggccctgggagagggccatttctcccaacaaggtgccctactatattaatcacgagacccagaccacttgttgggaccatcccaagatgacagaactgtaccagtccctggccgatctgaacaacgtgaggtttagcgcttacagaaccgctatgaagctgagacggctgcagaaggccctgtgcctggatctgctgtccctgtccgccgcctgcgatgccctggatcagcataatctgaagcagaacgatcagccaatggatatcctgcagatcatcaactgcctgaccactatctacgacaggctggagcaggagcacaacaacctggtgaacgtgcctctgtgcgtggatatgtgcctgaactggctgctgaacgtgtatgacactgggcgcaccggccggatcagagtgctgagttttaaaactgggattatctccctgtgtaaggcccacctggaggacaagtacaggtacctgttcaagcaggtggctagtagcactggattttgtgaccagcgccgcctgggactgctgctgcatgatagtatccagattcctagacagctgggagaggtggctagtttcggaggatctaacatcgaacccagcgtgcgcagctgtttccagtttgccaataacaaacctgaaatcgaggctgctctgttcctggattggatgcgcctggaaccacagagcatggtgtggctgcctgtgctgcacagagtggctgccgccgaaactgccaagcaccaggctaaatgcaacatctgcaaggaatgtcccattatcggctttcgctacaggagtctgaaacattttaactacgatatttgccagagctgcttcttttccggaagagtggccaaaggacacaagatgcactaccctatggtggaatattgcaccccaactacatctggcgaagatgtgcgcgattttgccaaggtgctgaagaataagtttcggactaagaggtacttcgccaagcacccccgcatggggtatctgccagtgcagacagtgctggaaggagacaatatggagaccgatacaatgtgagcggccgcaataaaagatctttattttcattagatctgtgtgttggttttttgtgtgtctagagcatggctacgtagataagtagcatggcgggttaatcattaactacaaggaacccctagtgatggagttggccactccctctctgcgcgctcgctcgctcactgaggccgggcgaccaaaggtcgcccgacgcccgggctttgcccgggcggcctcagtgagcgagcgagcgcgccagctggcgtaatagcgaagaggcccgcaccgatcgcccttcccaacagttgcgcagcctgaatggcgaatggaagttccagacgattgagcgtcaaaatgtaggtatttccatgagcgtttttcctgttgcaatggctggcggtaatattgttctggatattaccagcaaggccgatagtttgagttcttctactcaggcaagtgatgttattactaatcaaagaagtattgcgacaacggttaatttgcgtgatggacagactcttttactcggtggcctcactgattataaaaacacttctcaggattctggcgtaccgttcctgtctaaaatccctttaatcggcctcctgtttagctcccgctctgattctaacgaggaaagcacgttatacgtgctcgtcaaagcaaccatagtacgcgccctgtagcggcgcattaagcgcggcgggtgtggtggttacgcgcagcgtgaccgctacacttgccagcgccctagcgcccgctcctttcgctttcttcccttcctttctcgccacgttcgccggctttccccgtcaagctctaaatcgggggctccctttagggttccgatttagtgatttacggcacctcgaccccaaaaaacttgattagggtgatggttcacgtagtgggccatcgccctgatagacggtttttcgccctttgacgttggagtccacgttctttaatagtggactcttgttccaaactggaacaacactcaaccctatctcggtctattcttttgatttataagggattttgccgatttcggcctattggttaaaaaatgagctgatttaacaaaaatttaacgcgaattttaacaaaatattaacgtttacaatttaaatatttgcttatacaatcttcctgtttttggggcttttctgattatcaaccggggtacatatgattgacatgctagttttacgattaccgttcatcgattctcttgtttgctccagactctcaggcaatgacctgatagcctttgtagagacctctcaaaaatagctaccctctccggcatgaatttatcagctagaacggttgaatatcatattgatggtgatttgactgtctccggcctttctcacccgtttgaatctttacctacacattactcaggcattgcatttaaaatatatgagggttctaaaaatttttatccttgcgttgaaataaaggcttctcccgcaaaagtattacagggtcataatgtttttggtacaaccgatttagctttatgctctgaggctttattgcttaattttgctaattctttgccttgcctgtatgatttattggatgttggaagttcctgatgcggtattttctccttacgcatctgtgcggtatttcacaccgcatatggtgcactctcagtacaatctgctctgatgccgcatagttaagccagccccgacacccgccaacacccgctgacgcgccctgacgggcttgtctgctcccggcatccgcttacagacaagctgtgaccgtctccgggagctgcatgtgtcagaggttttcaccgtcatcaccgaaacgcgcgagacgaaagggcctcgtgatacgcctatttttataggttaatgtcatgataataatggtttcttagacgtcaggtggcacttttcggggaaatgtgcgcggaacccctatttgtttatttttctaaatacattcaaatatgtatccgctcatgagacaataaccctgataaatgcttcaataatattgaaaaaggaagagtatgagtattcaacatttccgtgtcgcccttattcccttttttgcggcattttgccttcctgtttttgctcacccagaaacgctggtgaaagtaaaagatgctgaagatcagttgggtgcacgagtgggttacatcgaactggatctcaacagcggtaagatccttgagagttttcgccccgaagaacgttttccaatgatgagcacttttaaagttctgctatgtggcgcggtattatcccgtattgacgccgggcaagagcaactcggtcgccgcatacactattctcagaatgacttggttgagtactcaccagtcacagaaaagcatcttacggatggcatgacagtaagagaattatgcagtgctgccataaccatgagtgataacactgcggccaacttacttctgacaacgatcggaggaccgaaggagctaaccgcttttttgcacaacatgggggatcatgtaactcgccttgatcgttgggaaccggagctgaatgaagccataccaaacgacgagcgtgacaccacgatgcctgtagcaatggcaacaacgttgcgcaaactattaactggcgaactacttactctagcttcccggcaacaattaatagactggatggaggcggataaagttgcaggaccacttctgcgctcggcccttccggctggctggtttattgctgataaatctggagccggtgagcgtgggtctcgcggtatcattgcagcactggggccagatggtaagccctcccgtatcgtagttatctacacgacggggagtcaggcaactatggatgaacgaaatagacagatcgctgagataggtgcctcactgattaagcattggtaactgtcagaccaagtttactcatatatactttagattgatttaaaacttcatttttaatttaaaaggatctaggtgaagatcctttttgataatctcatgaccaaaatcccttaacgtgagttttcgttccactgagcgtcagaccccgtagaaaagatcaaaggatcttcttgagatcctttttttctgcgcgtaatctgctgcttgcaaacaaaaaaaccaccgctaccagcggtggtttgtttgccggatcaagagctaccaactctttttccgaaggtaactggcttcagcagagcgcagataccaaatactgtccttctagtgtagccgtagttaggccaccacttcaagaactctgtagcaccgcgtacatacctcgctctgctaatcctgttaccagtggctgctgccagtggcgataagtcgtgtcttaccgggttggactcaagacgatagttaccggataaggcgcagcggtcgggctgaacggggggttcgtgcacacagcccagcttggagcgaacgacctacaccgaactgagatacctacagcgtgagctatgagaaagcgccacgcttcccgaagggagaaaggcggacaggtatccggtaagcggcagggtcggaacaggagagcgcacgagggagcttccagggggaaacgcctggtatctttatagtcctgtcgggtttcgccacctctgacttgagcgtcgatttttgtgatgctcgtcaggggggcggagcctatggaaaaacgccagcaacgcggcctttttacggttcctggccttttgctggccttttgctcacatgttctttcctgcgttatcccctgattctgtggataaccgtattaccgggtttgagtgagctgataccgctcgccgcagccgaacgaccgagcgcagcgagtcagtgagcgaccaagcggaagagc